European Patent Specification EP 3 518 658 B1, published May 6, 2026. Title: Parthenocarpic watermelon plants. Applicant: Nunhems B.V. The sequence listing filed with the application follows.

SEQUENCE LISTING (41 sequences)

SEQ ID NO: 1 - DNA, 151 bp, Citrullus lanatus
tagctttcaattagaatttcttatgaaaattgtttacgtatcaattatcattgtcattttgctagttttacctttaaagtttaattgatacaattgtaaatctcaccatgtttttcaaacgaaatctaaaagagtataaattgatacaatt

SEQ ID NO: 2 - DNA, 151 bp, Citrullus lanatus
agaagarggcgaagttgaggaaagagctcagagccctaagaagaggagcagaggaaattgctaaggacgcattgttcaacaaaaaggtgtgcagggtagtgcaacctgaagaagaaatacaaacgcatagacttcctgatcctcaagtaga

SEQ ID NO: 3 - DNA, 151 bp, Citrullus lanatus
taaaatggttgttcaaggaaggttattgaaagatgataatttgattttcaagtcaaacgataataggagacgcatcaaagaatcaaaagggatttttgagtgaaaattattatttaaaatgtttcctaattggttataaggatgtttttcc

SEQ ID NO: 4 - DNA, 151 bp, Citrullus lanatus
ccgagagcgagattctgagcgagagcgagagagcgagagtctgagcgagagagtgagattctggcgagggacttcccggaaagtagaatccgtcaaggcgagcggcgactgagagagagacaacgggaaacaaaggtaaagagagagtgtg

SEQ ID NO: 5 - DNA, 151 bp, Citrullus lanatus
aagcagcaggcattttagttaattaaacgaaaacttacgggaattaggattcattaacttaaattaactaaagttaattttaaaaaatagtggaattggtttaacttaagtttaattaactaattaaaaatataaaacttaatcagctttg

SEQ ID NO: 6 - DNA, 151 bp, Citrullus lanatus
aaaatttacctttagagtttggactcgctgccactggaaatcgactcactcactagcactgatctgagacttttacaaaaatggagaaagacttttacatgagttggtaacacatacggtgaccaactccaacaaacaatcatcgccttac

SEQ ID NO: 7 - DNA, 151 bp, Citrullus lanatus
cacctcttagatgcagggttgatagtttttggactcgtagtgcactagttagacgcctaattttcttcataaaggttctcaacttttcttaatttgagttctaaagtgattttcagtgagtaaagaagtgattccccgagtcttatttata

SEQ ID NO: 8 - DNA, 151 bp, Citrullus lanatus
aaatgaagttaaaccgaaaaaagtgtgctttcggagtagcttcaggcaagtttctaggcttcatggtcaatcatagaggaattaaagcaaatctagacaagatacgagctgtcctggagatggagtctcctaagacactaaagcaacttca

SEQ ID NO: 9 - DNA, 151 bp, Citrullus lanatus
aagggtgattgtacaagagaaggatttgtagctaagaatggacataaggaaagagagaggacgcatgatagtatgcgattaaggcagacgcatggtattatatggtaagctgaaacgtatagtagtatgcgtttaagacttaaacacctag

SEQ ID NO: 10 - DNA, 151 bp, Citrullus lanatus
atgtttgattgaaaccaaaaaccagaagaattcgaagctcaacccaatcccaagaaagaggagttggaagtggtgaaaacgggagaagaagaagaagaacaacaacaacaacaagatgctgaatcttactgttcgaagtttactgggtaga

SEQ ID NO: 11 - DNA, 151 bp, Citrullus lanatus
gtttggtgaatatctgaaacatacaaaatggatttaattgtgtagataaattcattgtttagaaactttcaaattgaattgaaatttcaaattaaaatgatgtttcatgtacaaatttaacatgtatgaaagttaaatttgtagtttcttc

SEQ ID NO: 12 - DNA, 151 bp, Citrullus lanatus
  misc_feature (146)..(146): n is a, c, g, or t
ttttgttatctactttctaaaagtgttctaaaaaaccaatcaatggtttggaaactagttttcaaaaatttatttttgtttttaaaaatttgacgaaaaattcaaaagtttctttaagaaaggttgaagctatagtaaagaatttntgagg

SEQ ID NO: 13 - DNA, 151 bp, Citrullus lanatus
caaaagttgcatgatatagtaatagccaaacacataatgtaatgttaagtatccgaaggtcgtagtaattctcttgacttacattaacagcaacaatggaaggaaaaaaaaacccaaataagtacccaaaaattaaagaatactttctatg

SEQ ID NO: 14 - DNA, 151 bp, Citrullus lanatus
ttgtagaaattaaacccacaaatgatagaaatcgaactctcacatttgtacgattattacaatttgtacaattatattagtctgagagttcaattttaacatttgtataagtttgaagtctcaatttttaaaattaaaagtttaaggggat

SEQ ID NO: 15 - DNA, 151 bp, Citrullus lanatus
tggagtcacccttcgtcggccatattctcgcatttccccgtcactcagttgcagcgctccagccttcacggtgcggccttaatcgcagttcacagcattgtggcatcgtcatagttgtcgcgccgcagcatcttggtcgtcgcgccccagc

SEQ ID NO: 16 - DNA, 151 bp, Citrullus lanatus
acttttctaaaaaacaaccattacttatgcaatatgattgattcctaatttcttgaaaccaagttaataagcataacattaagattagtcatgatcaactttttctaataacctagctatttaattaatagagattcaatgctatagatcc

SEQ ID NO: 17 - DNA, 151 bp, Citrullus lanatus
atgtaattagagtaagtatccatatgaaatatgatccaatcgatatttgaaataattaacaaacttgctactaaagaaaactttagcttttaaacctacacaaatttaatatatgaaatacacttttgatctggttgaattccaattctaa

SEQ ID NO: 18 - DNA, 151 bp, Citrullus lanatus
tttactcaaattttaaaaaacttgttttgtttttagaacggtgaaaattaccataatttaaaaattggaaggaaccaatataaatttttaaggaaaaaaaaacaaaaaaattaaaacaaaatcgttgcaaaaagacctttaattatattga

SEQ ID NO: 19 - DNA, 151 bp, Citrullus lanatus
tctaccaatcttactctattaattctcccaatttttattagaaaaattctaagaaaattcttattcccataagcggttcccacaaaccagatctttgcgcgagtcatagcgaggaagatctcttggaaaagaaagactacaaggagaagac

SEQ ID NO: 20 - DNA, 151 bp, Citrullus lanatus
aacattttactataaattttggaaacacattcacatattatatttctttacataaaaattattgttgttatttaatcaatttcaataaaaattaactttgagagactaaatttaagatttattaaaaatacataaattaaaattggacaat

SEQ ID NO: 21 - DNA, 151 bp, Citrullus lanatus
aacatcctaaaactatgagtttagccacggatagacatcaaatacatacattcatatgagttctcaagcataaaagtaaaagagaaagagaaacttaggaagaaagactctcgaattgcttccccgcgttgaattccttcgatctccactt

SEQ ID NO: 22 - DNA, 151 bp, Citrullus lanatus
cttttcaggtggctactcctaaacatttctttacaggtgggtgcttctagcatgacagttttacgtagtatttggcagagttactggctcgataagcatggggatgccatggagagcgttgttgatcagcttgcacgaagtctatcagaga

SEQ ID NO: 23 - DNA, 151 bp, Citrullus lanatus
atatgtcattaataaattgctaactagactaaaaatttagatgtctaaacacatatgttgcttaggtgtgccaaataatcggattgatatatatggaaatttacgatcatagaataattattttagggccatttttttaattgacgtttaa

SEQ ID NO: 24 - DNA, 151 bp, Citrullus lanatus
tcagatgagtgacgttcaatttgtctattttattgtacaatcaatgatcacaacaaagctatttatattttcaatcattctatttttgttgtatagtaattttgttatatagtaatttcgttatcctaaactattttcattcttctaagta

SEQ ID NO: 25 - DNA, 5135 bp, Citrullus lanatus
  exon (1018)..(2088)
  CDS (1018)..(2088)
  Intron (2089)..(2185)
  exon (2186)..(2353)
  CDS (2186)..(2353)
  Intron (2354)..(3098)
  exon (3099)..(3265)
  CDS (3099)..(3265)
  Intron (3266)..(4324)
  exon (4325)..(4607)
  CDS (4325)..(4604)
aaacattcatacttttgaagaaaattagtatattatttatttatattatatttacagattatttattgattattttttaaatatttattgaattttttataatataataaaaatgtcgacatgtcaacacaaaattaatttcatattatgaattagaagtagggaataagagtatgtttggaataaattttcaagtatttaattttaaaaataagtcacttcaaaagaaatataagtgtttggcaaccactcaaactgtattttaaaagccattagtgtctttattataaatacttttcttatcaaaagtgtttaaatgaaaataaaagtttgaagacatttcttttctaggttaatcgaatggcttctaaatttaagatttatcaaatgtatatggtatgtttggttcaaaagagtttttgagcttataattaaagaacatcaatctcatgacttatcaattttttgtaatgtgtatttaaaaaaaaaaagaaataaaaaagaaaaagaaaagaaaaacattttgtaataggaccctacaattaaacaatttaggacatgtctagggagtgattctaaaatagttaaatccacttttgttattattgaaatcacttttaaatatttcaaatcttccaaacacaaaatttattatataaaaattatacttaaaaatgtaaaattaaatactaaattaatttggagtgatttaatatatgttttggggatatatccatttcaaaatcactccaaatatgaatttcataaaattaaagttgaatatttgaaagtagaagactaaaatggaaaagaatatagaggtgaggggccaaaatgatatttaactaaataattattattatttattagattagcacgagaggaggtgacagtgagggaccctctccaaaaaaaaaaaaaactcacttccaattcacaattctcttttgcttcctaacttccataactgctctgctttccatcacgaaactcatcttcatcttcttcattcgaacaatgaagtccaagaagccaagggcaaatcccaaacccgaatcctactctccgccgaagaagaagctccgttctcagcttccacggcgcagacgctctcggatttctccttttttctgctccttggactccgattcccctgctccttctaccaccattgcttttgcttcttcttcctttgctgccgccgaatccagctccacttccttccacgcaggcggacctgaggtttctagccagctcaacgcgtgttttggattccagaggccgaatttgcggaagagacgatttggttcgggtggtgttaatttggatgaagtttcgaagaaggaggttggagtagggagtaatgtggaagtgtctgaatcgtcttgcgttgaatcaaattctggagttgattttggtgttctcggaccaagcactagctccaggttgaagattagaagtgattttaggagaactattgacgaaaatgaagatccaatcgatcaagcggataatggagttgtgaagtttcaattgacggatgctgatgtctcgtcgaagctttgtgaaaagggagctgtgccactcactccttgtggagagtcttgcgctgagtctatcttccagagcgtttgttcgttcgaagagaaaggattagacgttgaagaaaacagactatgggaatttcagttaccagaactaccgagaaatgagatcaatgaaactttcactgtttcgaagtcggattcgacgatagaacagtggcctaatagcttgaagtttgaatcggatcttgcttgcacggagcaattctcttatgagaatgtttcggaatactctagccaggcgttgtccgagcttcaatcaacaattctattggagacgtctgatactgactgctcagattacactccttcaatttttttggaatccggaagcgaattttcagagaaatcgaacgacgacgcagctccttcgtcaacatttagcatgttgctgcagtacagacgcgactttctaaacttaaatgcctctccagacatcagaactagctcgtctattgaagaagagaaagtagatcaatctacggtaattcgctatcttcatgcttccttgacgtttcatttgcaacaaacctgaagctaatcaaacaactatatatatatattatttgattttaaattagattttgagatttgaagaattggacgatgaagaagcctatctaatgttcagaagtagagaaagacgccaattgattattcgcgactacgtagaggagtatcggtccacaacggattatggcgatctcattctccagcaacggtcaaatgtggtccaatggatagttgaagtaagtccttgataccaaaccaccgtgtttctctcaataattcctgaattagcatgagatattttgctccggttttccattttcatcgttaatagcattggtattctgagacattggaactgtttagtgtatcgaggtagtttgaagcactgactctcatatttcaatttgcactgaatcgctaattagttcttaacatctcataaaatgagttcccttgccttatttgctatggaactttatccgacagcgtacttttctgatttggctatcccaacaatgtgatttactaatgaaaattacaaagtcattaccatgatcatactttccactacttaaaagccagcagtttatgatcttgcacctgttacatctagttgttataagctcattctaacgaatgaggcctgccaccagcacaacgcatctggcatcttgaatcaactaagtttaactgatttttcatttcttttcttacttctgcttgaatatattttctgtttgtttttcatcttaataatagaatacagattcataaccgcgagatttgtgcttattactgtggatgttgacattttcttaggaatactccaatgtagttgcattttcatcatctgttgacgtttctagttcaaggaatacattctttatactatttttattccttttctgcgttaatacttgtcaccaaccaattgggtcaaattttttacattatgttgctttgttttgttgaatgatgcagcgatcgagagattccaaacttcatcaggagacgacatttttaggagttaccctcctggaccagattctgagcagaggattcttcaaagctggaagacaccttcaaattctgggcatagcatgtctaactttggcgactagaattgaagaaaatcagtcatacagctggtgactttttttctatcttttgtctatttgtgtgcatctcagttttaactatataacaagtgttgttcttatctactgtaacttcaacttaacttcgttagtatgatgaatattgcttgaaaacaaactgtatgccagttggtcttcttgtttcgatccaagggagtgaaattgggtaagttaggatcgaatgctaagtagtactagaaataataatcagaaagaattgtattaaagtaattgaatctaatagtcttgaatattttttctaaagttcaaagtgtcgagcctgaaagctttgcgtttacatggaccaaagtaatgttgtgaatatatcgtaggtcctcttatagcaattatgtaacaaataatagccatacattagtgtcgatacacaccacccgtacggtactgtagtcgaatattgccataacactatctttcagttcttatgttaacaattcatgtgcacagaagagacccgagacccaccaagaaaacattatctttgacttgtatatagaactctaagtcgagtcaaatgtaaaacaattctttttcttctcttctctttctcaaacttccttttgtagccttcatttatctttgacttgcaatttacatgcaaaatgttaaataattgtgatttgtttaattaaatagagccttgtgaattgagaaggtatccaagctagctggtgggtctcgagcttggtggatatatttataaagctatgataggactgatttgttttatttttgggcatttcagggtgcagcaaaggaatatccgtgtagagagcaacacgtacagaagatctgaagttgttggcatggaatggcttgttgaagaagtcttaaagttccattgtttcttgccaactgtttacaacttcttatggtacatcttcctttgactaacttgaccattggtgggaagggaaaaagttttccctttcgtgcatccattttcaataaactccttccgcccattaacaatttgaatctactgcgaataacatgctttatttaattttctttttttgaaaattatcttaggttctacctgaaagctgctggagctgactcgaatttggagaatcgagctaagaactttgcggagctggttctttcagacaaagtccaattttgttatttcccttcaactattgcagctgcggttgtcatcttggcgtccctaggagaaaaacaagatgcaccaagtcaacgagtcattgaggtacataaatacaaatacctgttagagagaaaactcctttatctttatattgacccaattgaacaaataaacaagtattttgaaatcgagaagaaactttaaagttttacaaaaacaccataatctaaatccaattagattcaactgtaatgtaaagtacaataataaaatacatataccataaggaaatggtaggttatagtgtttgtttcaattagatattcaatttatatattagttagtgttgttaatctccctgaatatttcttactaacttgaggaaggtctcctgtcttctggaaacccttccatgcccaaaatttcagccttctgctattcccattaagtcaaacatgtaatgagtttacttttctttctccttctaattattaattatttttaataatttatttgtctaattcattttctgtagtctgaacccacgaacttgcttatcacaaaatccaaaaccaaaaaccccatcacaattttggaaatctttttgagaactgctactataaccatgtaatttctttcaaaatctacaaaaatagaaataacacttatttagactatctgtggtactatctcataacatctggtgcattgtggctttgcagacgcatgtca

SEQ ID NO: 26 - protein, 562 aa, Citrullus lanatus
MKSKKPRANPKPESYSPPKKKLRSQLPRRRRSRISPFFCSLDSDSPAPSTTIAFASSSFAAAESSSTSFHAGGPEVSSQLNACFGFQRPNLRKRRFGSGGVNLDEVSKKEVGVGSNVEVSESSCVESNSGVDFGVLGPSTSSRLKIRSDFRRTIDENEDPIDQADNGVVKFQLTDADVSSKLCEKGAVPLTPCGESCAESIFQSVCSFEEKGLDVEENRLWEFQLPELPRNEINETFTVSKSDSTIEQWPNSLKFESDLACTEQFSYENVSEYSSQALSELQSTILLETSDTDCSDYTPSIFLESGSEFSEKSNDDAAPSSTFSMLLQYRRDFLNLNASPDIRTSSSIEEEKVDQSTILRFEELDDEEAYLMFRSRERRQLIIRDYVEEYRSTTDYGDLILQQRSNVVQWIVERSRDSKLHQETTFLGVTLLDQILSRGFFKAGRHLQILGIACLTLATRIEENQSYSWFYLKAAGADSNLENRAKNFAELVLSDKVQFCYFPSTIAAAVVILASLGEKQDAPSQRVIEVHKYKYLLERKLLYLYIDPIEQINKYFEIEKKL

SEQ ID NO: 27 - RNA, 1673 nt, Artificial Sequence
  Induced by mutation
  mRNA (1)..(1673)
  CDS (1)..(1098)
augaaguccaagaagccaagggcaaaucccaaacccgaauccuacucuccgccgaagaagaagcuccguucucagcuuccacggcgcagacgcucucggauuucuccuuuuuucugcuccuuggacuccgauuccccugcuccuucuaccaccauugcuuuugcuucuucuuccuuugcugccgccgaauccagcuccacuuccuuccacgcaggcggaccugagguuucuagccagcucaacgcguguuuuggauuccagaggccgaauuugcggaagagacgauuugguucgggugguguuaauuuggaugaaguuucgaagaaggagguuggaguagggaguaauguggaagugucugaaucgucuugcguugaaucaaauucuggaguugauuuugguguucucggaccaagcacuagcuccagguugaagauuagaagugauuuuaggagaacuauugacgaaaaugaagauccaaucgaucaagcggauaauggaguugugaaguuucaauugacggaugcugaugucucgucgaagcuuugugaaaagggagcugugccacucacuccuuguggagagucuugcgcugagucuaucuuccagagcguuuguucguucgaagagaaaggauuagacguugaagaaaacagacuaugggaauuucaguuaccagaacuaccgagaaaugagaucaaugaaacuuucacuguuucgaagucggauucgacgauagaacaguggccuaauagcuugaaguuugaaucggaucuugcuugcacggagcaauucucuuaugagaauguuucggaauacucuagccaggcguuguccgagcuucaaucaacaauucuauuggagacgucugauacugacugcucagauuacacuccuucaauuuuuuuggaauccggaagcgaauuuucagagaaaucgaacgacgacgcagcuccuucgucaacauuuagcauguugcugcaguacagacgcgacuuucuaaacuuaaaugccucuccagacaucagaacuagcucgucuauugaagaagagaaaguagaucaaucuacgaauuggacgaugaagaagccuaucuaauguucagaaguagagaaagacgccaauugauuauucgcgacuacguagaggaguaucgguccacaacggauuauggcgaucucauucuccagcaacggucaaaugugguccaauggauaguugaacgaucgagagauuccaaacuucaucaggagacgacauuuuuaggaguuacccuccuggaccagauucugagcagaggauucuucaaagcuggaagacaccuucaaauucugggcauagcaugucuaacuuuggcgacuagaauugaagaaaaucagucauacagcugguucuaccugaaagcugcuggagcugacucgaauuuggagaaucgagcuaagaacuuugcggagcugguucuuucagacaaaguccaauuuuguuauuucccuucaacuauugcagcugcgguugucaucuuggcgucccuaggagaaaaacaagaugcaccaagucaacgagucauugagguacauaaauacaaauaccuguuagagagaaaacuccuuuaucuuuauauugacccaauugaacaaauaaacaaguauuuugaaaucgagaagaaacuuuaa

SEQ ID NO: 28 - protein, 365 aa, Artificial Sequence
  Synthetic Construct
MKSKKPRANPKPESYSPPKKKLRSQLPRRRRSRISPFFCSLDSDSPAPSTTIAFASSSFAAAESSSTSFHAGGPEVSSQLNACFGFQRPNLRKRRFGSGGVNLDEVSKKEVGVGSNVEVSESSCVESNSGVDFGVLGPSTSSRLKIRSDFRRTIDENEDPIDQADNGVVKFQLTDADVSSKLCEKGAVPLTPCGESCAESIFQSVCSFEEKGLDVEENRLWEFQLPELPRNEINETFTVSKSDSTIEQWPNSLKFESDLACTEQFSYENVSEYSSQALSELQSTILLETSDTDCSDYTPSIFLESGSEFSEKSNDDAAPSSTFSMLLQYRRDFLNLNASPDIRTSSSIEEEKVDQSTNWTMKKPI

SEQ ID NO: 29 - DNA, 151 bp, Citrullus lanatus
attggtttgtgactcggattcagaggaattgttattggaagagaagctatcatttatgcatgaaacgaggcatgcattcggaaggactgccctgctcttaagtggaggtgcttcacttggagcttttcatacaggagttgtcaaaactctg

SEQ ID NO: 30 - DNA, 906 bp, Citrullus lanatus
atgagggaagaacactcgaattggttctctaggtgggaagaggagcttccatctccagatgaattgatgcctctttctcaaaccctaataacccccgatctagctttggcctttgatattcagaatcccagcaatagcagtccgccgttgccttgtccatctccgccgctttcgaatcctctgcctggctctggcaacggaattgcgcagcccaactcggcggatttcggcgattctgccgatttgggctccggcgccgccagcgacgagccggctcggaccctcaagcgaccacgccttgtttggacgcctcagctccacaagcgattcgtcgatgctgttgctcatttagggataaaaaatgccgtccccaagaccataatgcagctcatgagtgtcgatggcttgacccgagagaacgtagctaaccatttgcagaagtaccgcctctatctcaagcggatgcaggggttgtcctccggcggcggcggtggtggtggtggcttggttgcttcctccgatcccgccactgaccatttgtttgccagctccccagttccaccccatttgcttcactctgctcgcaccagttcagaccatttcttgccctttgttcccatggccactctgcagcagcaccaccatcaccagcagcagatggccgctgctgctgctgtcgccgtccatccgcagctccagccgccttatcatcggcaggtcgggcatttcgggtcaccgccgaatggccagtttgagcatccatttttagctagacagtcccagcctatccatagaatgggagcaccagtgcctaattcagttcctaattacatagaggatttggaatcagccaatgccagtggaggaagaaaagttctcaccttatttcctactggggatgattga

SEQ ID NO: 31 - protein, 301 aa, Citrullus lanatus mutant wop1 protein
MREEHSNWFSRWEEELPSPDELMPLSQTLITPDLALAFDIQNPSNSSPPLPCPSPPLSNPLPGSGNGIAQPNSADFGDSADLGSGAASDEPARTLKRPRLVWTPQLHKRFVDAVAHLGIKNAVPKTIMQLMSVDGLTRENVANHLQKYRLYLKRMQGLSSGGGGGGGGLVASSDPATDHLFASSPVPPHLLHSARTSSDHFLPFVPMATLQQHHHHQQQMAAAAAVAVHPQLQPPYHRQVGHFGSPPNGQFEHPFLARQSQPIHRMGAPVPNSVPNYIEDLESANASGGRKVLTLFPTGDD

SEQ ID NO: 32 - protein, 301 aa, Citrullus lanatus wild type WOP1 protein
MREEHSNWFSRWEEELPSPDELMPLSQTLITPDLALAFDIQNPSNSSPPLPCPSPPLSNPLPGSGNGIAQPNSADFGDSADLGSGAASDEPARTLKRPRLVWTPQLHKRFVDAVAHLGIKNAVPKTIMQLMSVDGLTRENVASHLQKYRLYLKRMQGLSSGGGGGGGGLVASSDPATDHLFASSPVPPHLLHSARTSSDHFLPFVPMATLQQHHHHQQQMAAAAAVAVHPQLQPPYHRQVGHFGSPPNGQFEHPFLARQSQPIHRMGAPVPNSVPNYIEDLESANASGGRKVLTLFPTGDD

SEQ ID NO: 33 - protein, 301 aa, Cucumis sativus
MREEHSNWFSRWEDELPSPDELMPLSQTLITPDLALAFDIQNPSNSSPPLPCPSPPLSNPLPGSGNGIVPPNSADFGDSADLGSGAASDEPARTLKRPRLVWTPQLHKRFVDAVAHLGIKNAVPKTIMQLMSVDGLTRENVASHLQKYRLYLKRMQGLSGGGGGGGAALVGSSDPATDHLFASSPVPPHLLHSARTSSDHFLPYVPMATLQQHHHHQQQMAAAAAVAGHTQLQPPYHRQVGHFGSPPNGQFEHPFLARQSQPIHRMGTPVHNSVPNYIEDLESANATGGRKVLTLFPTGDD

SEQ ID NO: 34 - protein, 301 aa, Cucumis melo
MREEHSNWFSRWEEELPSPDELMPLSQTLITPDLALAFDIQNPSNSSPPLPCPSPPLSNPLPGSGNGIVPPNSADFGDSADLGSGAASDEPARTLKRPRLVWTPQLHKRFVDAVAHLGIKNAVPKTIMQLMSVDGLTRENVASHLQKYRLYLKRMQGLSGGGAGGGAALVGSSDPATDHLFASSPVPPHLLHSARTSSDHFLPFVPMATLQQHHHHQQQMAAAAAVAGHTQLQPPYHRQVGHFGSPPNGQFEHPFLARQSQPIHRMGTSVHNSVPNYIEDLESANATGGRKVLTLFPTGDD

SEQ ID NO: 35 - protein, 54 aa, artificial
  myb-like DNA binding domain SHAQKYF
RPRLVWTPQLHKRFVDAVAHLGIKNAVPKTIMQLMSVDGLTRENVASHLQKYRL

SEQ ID NO: 36 - DNA, 39 bp, artificial
  PCR primer
cctacacgacgctcttccaagaggagcttccatctccag

SEQ ID NO: 37 - DNA, 37 bp, artificial
  PCR primer
ctgctgaaccgctcttccagcccaaatcggcagaatc

SEQ ID NO: 38 - DNA, 213 bp, artificial
  amplified fragment
aagaggagcttccatctccagatgaattgatgcctctttctcaaaccctaataacccccgatctagctttggcctttgatattcagaatcccagcaatagcagtccgccgttgccttgtccatctccgccgctttcgaatcctctgcctggctctggcaacggaattgcgcagcccaactcggcggatttcggcgattctgccgatttgggct

SEQ ID NO: 39 - DNA, 37 bp, artificial
  PCR primer
cctacacgacgctcttccgtggcttggttgcttcctc

SEQ ID NO: 40 - DNA, 37 bp, artificial
  PCR primer
ctgctgaaccgctcttccgatgataaggcggctggag

SEQ ID NO: 41 - DNA, 213 bp, artificial
  ampliefied PCR fragment
gtggcttggttgcttcctccgatcccgccactgaccatttgtttgccagctccccagttccaccccatttgcttcactctgctcgcaccagttcagaccatttcttgccctttgttcccatggccactctgcagcagcaccaccatcaccagcagcagatggccgctgctgctgctgtcgccgtccatccgcagctccagccgccttatcatc